European Patent Specification EP 4 053 291 B1, published May 1, 2024. Title: ISOTHERMAL AMPLIFICATION COMPONENTS AND PROCESSES. Applicant: NAT DIAGNOSTICS, INC. The sequence listing filed with the application follows.

SEQUENCE LISTING (12 sequences)

SEQ ID NO: 1 - DNA, 11 bp, Artificial Sequence
  source: /note="Description of Artificial Sequence: Synthetic oligonucleotide"
ggcttatggag

SEQ ID NO: 2 - DNA, 10 bp, Artificial Sequence
  source: /note="Description of Artificial Sequence: Synthetic oligonucleotide"
ataccgctta

SEQ ID NO: 3 - DNA, 10 bp, Artificial Sequence
  source: /note="Description of Artificial Sequence: Synthetic oligonucleotide"
gcttatggag

SEQ ID NO: 4 - DNA, 28 bp, Artificial Sequence
  source: /note="Description of Artificial Sequence: Synthetic oligonucleotide"
ctggctaccgcttaactccataagccag

SEQ ID NO: 5 - DNA, 10 bp, Artificial Sequence
  source: /note="Description of Artificial Sequence: Synthetic oligonucleotide"
aggcttatgg

SEQ ID NO: 6 - DNA, 10 bp, Artificial Sequence
  source: /note="Description of Artificial Sequence: Synthetic oligonucleotide"
ttataccgct

SEQ ID NO: 7 - DNA, 29 bp, Artificial Sequence
  source: /note="Description of Artificial Sequence: Synthetic oligonucleotide"
  misc_feature (26)..(29): /note="Phosphorothioate linkage"
ccgcgagccttataccgcttaactcgcgg

SEQ ID NO: 8 - protein, 775 aa, Artificial Sequence
  source: /note="Description of Artificial Sequence: Synthetically derived Thermococcus sp. strain 9 degrees N-7 polypeptide"
MILDTDYITENGKPVIRVFKKENGEFKIEYDRTFEPYFYALLKDDSAIEDVKKVTAKRHGTVVKVKRAEKVQKKFLGRPIEVWKLYFNHPQDVPAIRDRIRAHPAVVDIYEYDIPFAKRYLIDKGLIPMEGDEELTMLAFDIETLYHEGEEFGTGPILMISYADGSEARVITWKKIDLPYVDVVSTEKEMIKRFLRVVREKDPDVLITYNGDNFDFAYLKKRCEELGIKFTLGRDGSEPKIQRMGDRFAVEVKGRIHFDLYPVIRRTINLPTYTLEAVYEAVFGKPKEKVYAEEIAQAWESGEGLERVARYSMEDAKVTYELGREFFPMEAQLSRLIGQSLWDVSRSSTGNLVEWFLLRKAYKRNELAPNKPDERELARRRGGYAGGYVKEPERGLWDNIVYLDFRSLYPSIIITHNVSPDTLNREGCKEYDVAPEVGHKFCKDFPGFIPSLLGDLLEERQKIKRKMKATVDPLEKKLLDYRQRAIKILANSFYGYYGYAKARWYCKECAESVTAWGREYIEMVIRELEEKFGFKVLYADTDGLHATIPGADAETVKKKAKEFLKYINPKLPGLLELEYEGFYVRGFFVTKKKYAVIDEEGKITTRGLEIVRRDWSEIAKETQARVLEAILKHGDVEEAVRIVKEVTEKLSKYEVPPEKLVIHEQITRDLRDYKATGPHVAVAKRLAARGVKIRPGTVISYIVLKGSGRIGDRAIPADEFDPTKHRYDAEYYIENQVLPAVERILKAFGYRKEDLRYQKTKQVGLGAWLKVKGKK

SEQ ID NO: 9 - protein, 775 aa, Artificial Sequence
  source: /note="Description of Artificial Sequence: Synthetically derived Thermococcus sp. strain 9 degrees N-7 polypeptide"
MILDTDYITENGKPVIRVFKKENGEFKIEYDRTFEPYFYALLKDDSAIEDVKKVTAKRHGTVVKVKRAEKVQKKFLGRPIEVWKLYFNHPQDVPAIRDRIRAHPAVVDIYEYDIPFAKRYLIDKGLIPMEGDEELTMLAFDIDTLYHEGEEFGTGPILMISYADGSEARVITWKKIDLPYVDVVSTEKEMIKRFLRVVREKDPDVLITYNGDNFDFAYLKKRCEELGIKFTLGRDGSEPKIQRMGDRFAVEVKGRIHFDLYPVIRRTINLPTYTLEAVYEAVFGKPKEKVYAEEIAQAWESGEGLERVARYSMEDAKVTYELGREFFPMEAQLSRLIGQSLWDVSRSSTGNLVEWFLLRKAYKRNELAPNKPDERELARRRGGYAGGYVKEPERGLWDNIVYLDFRSLYPSIIITHNVSPDTLNREGCKEYDVAPEVGHKFCKDFPGFIPSLLGDLLEERQKIKRKMKATVDPLEKKLLDYRQRAIKILANSFYGYYGYAKARWYCKECAESVTAWGREYIEMVIRELEEKFGFKVLYADTDGLHATIPGADAETVKKKAKEFLKYINPKLPGLLELEYEGFYVRGFFVTKKKYAVIDEEGKITTRGLEIVRRDWSEIAKETQARVLEAILKHGDVEEAVRIVKEVTEKLSKYEVPPEKLVIHEQITRDLRDYKATGPHVAVAKRLAARGVKIRPGTVISYIVLKGSGRIGDRAIPADEFDPTKHRYDAEYYIENQVLPAVERILKAFGYRKEDLRYQKTKQVGLGAWLKVKGKK

SEQ ID NO: 10 - DNA, 12 bp, Artificial Sequence
  source: /note="Description of Artificial Sequence: Synthetic oligonucleotide"
atgcatgcatgc

SEQ ID NO: 11 - DNA, 12 bp, Artificial Sequence
  source: /note="Description of Artificial Sequence: Synthetic oligonucleotide"
gcatgcatgcat

SEQ ID NO: 12 - DNA, 18 bp, Artificial Sequence
  source: /note="Description of Artificial Sequence: Synthetic oligonucleotide"
atgcataaaaaagcatgc